European Patent Application EP 4 129 311 A1, published February 8, 2023. Title: Genome-edited pluripotent stem cell-based therapeutic agent. Applicant: Keio University. The sequence listing filed with the application follows.

SEQUENCE LISTING (44 sequences)

SEQ ID NO: 1 - DNA, 34 bp, Artificial Sequence
  loxP
ataacttcgtatagcatacattatacgaagttat

SEQ ID NO: 2 - DNA, 34 bp, Artificial Sequence
  lox71
taccgttcgtatagcatacattatacgaagttat

SEQ ID NO: 3 - DNA, 34 bp, Artificial Sequence
  lox66
ataacttcgtatagcatacattatacgaacggta

SEQ ID NO: 4 - DNA, 34 bp, Artificial Sequence
  lox2272
ataacttcgtataggatactttatacgaagttat

SEQ ID NO: 5 - DNA, 19 bp, Artificial Sequence
  primer
gacgtggaggaaaatcccg

SEQ ID NO: 6 - DNA, 19 bp, Artificial Sequence
  primer
gggtcggatctaccgttcg

SEQ ID NO: 7 - DNA, 20 bp, Artificial Sequence
  primer
ccctggagaagagctacgag

SEQ ID NO: 8 - DNA, 20 bp, Artificial Sequence
  primer
cgggattttcctccacgtca

SEQ ID NO: 9 - DNA, 22 bp, Artificial Sequence
  primer
aagtcttctaacatgcggtgac

SEQ ID NO: 10 - DNA, 20 bp, Artificial Sequence
  primer
ggtgtacagagtggtgtcct

SEQ ID NO: 11 - DNA, 20 bp, Artificial Sequence
  primer
cagccatgtacgttgctatc

SEQ ID NO: 12 - DNA, 20 bp, Artificial Sequence
  primer
attttcctccacgtcaccgc

SEQ ID NO: 13 - DNA, 22 bp, Artificial Sequence
  primer
aggaagtcttctaacatgcggt

SEQ ID NO: 14 - DNA, 19 bp, Artificial Sequence
  primer
ggtcggatctaccgttcgt

SEQ ID NO: 15 - DNA, 21 bp, Artificial Sequence
  primer
ttctaacatgcggtgacgtgg

SEQ ID NO: 16 - DNA, 21 bp, Artificial Sequence
  primer
gtcagtctccacaatctgctt

SEQ ID NO: 17 - DNA, 23 bp, Artificial Sequence
  primer
gcagaggaagtcttctaacatgc

SEQ ID NO: 18 - DNA, 21 bp, Artificial Sequence
  primer
aagggacttcctgtaacaacg

SEQ ID NO: 19 - DNA, 19 bp, Artificial Sequence
  primer
ctggcatcgtgatggactc

SEQ ID NO: 20 - DNA, 23 bp, Artificial Sequence
  primer
acacttggcctcatttttaaggt

SEQ ID NO: 21 - DNA, 20 bp, Artificial Sequence
  primer
aagtactccgtgtggatcgg

SEQ ID NO: 22 - DNA, 24 bp, Artificial Sequence
  primer
gtcacacttggcctcatttttaag

SEQ ID NO: 23 - DNA, 21 bp, Artificial Sequence
  primer
tccatcatgaagtgtgacgtg

SEQ ID NO: 24 - DNA, 24 bp, Artificial Sequence
  primer
tcacacttggcctcatttttaagg

SEQ ID NO: 25 - DNA, 19 bp, Artificial Sequence
  primer
gacgtggaggaaaatcccg

SEQ ID NO: 26 - DNA, 20 bp, Artificial Sequence
  primer
gggtcggatccataacttcg

SEQ ID NO: 27 - DNA, 20 bp, Artificial Sequence
  primer
ccctggagaagagctacgag

SEQ ID NO: 28 - DNA, 20 bp, Artificial Sequence
  primer
cgggattttcctccacgtca

SEQ ID NO: 29 - DNA, 22 bp, Artificial Sequence
  primer
aagtcttctaacatgcggtgac

SEQ ID NO: 30 - DNA, 20 bp, Artificial Sequence
  primer
ggtgtacagagtggtgtcct

SEQ ID NO: 31 - DNA, 20 bp, Artificial Sequence
  primer
cagccatgtacgttgctatc

SEQ ID NO: 32 - DNA, 20 bp, Artificial Sequence
  primer
attttcctccacgtcaccgc

SEQ ID NO: 33 - DNA, 22 bp, Artificial Sequence
  primer
aggaagtcttctaacatgcggt

SEQ ID NO: 34 - DNA, 20 bp, Artificial Sequence<220><223>  primer
ggtcggatccataacttcgt

SEQ ID NO: 35 - DNA, 21 bp, Artificial Sequence
  primer
ttctaacatgcggtgacgtgg

SEQ ID NO: 36 - DNA, 21 bp, Artificial Sequence
  primer
gtcagtctccacaatctgctt

SEQ ID NO: 37 - DNA, 23 bp, Artificial Sequence
  primer
gcagaggaagtcttctaacatgc

SEQ ID NO: 38 - DNA, 21 bp, Artificial Sequence
  primer
aagggacttcctgtaacaacg

SEQ ID NO: 39 - DNA, 19 bp, Artificial Sequence
  primer
ctggcatcgtgatggactc

SEQ ID NO: 40 - DNA, 23 bp, Artificial Sequence
  primer
acacttggcctcatttttaaggt

SEQ ID NO: 41 - DNA, 20 bp, Artificial Sequence
  primer
aagtactccgtgtggatcgg

SEQ ID NO: 42 - DNA, 24 bp, Artificial Sequence
  primer
gtcacacttggcctcatttttaag

SEQ ID NO: 43 - DNA, 21 bp, Artificial Sequence
  primer
tccatcatgaagtgtgacgtg

SEQ ID NO: 44 - DNA, 24 bp, Artificial Sequence
  primer
tcacacttggcctcatttttaagg